European Patent Specification EP 3 957 733 B1, published January 15, 2025. Title: Simple detection method of nucleic acid sequence. Applicant: Nihon University. The sequence listing filed with the application follows.

SEQUENCE LISTING (27 sequences)

SEQ ID NO: 1 - DNA, 18 bp, Artificial Sequence
  P1
ggatcaggccatttttgg

SEQ ID NO: 2 - DNA, 18 bp, Artificial Sequence
  P2
gaagctgttgttatcact

SEQ ID NO: 3 - DNA, 67 bp, Artificial Sequence
  cT1
ccccaaaaaggagcttgaggttctcctttaaaaagaagctgttgtattgttgtcgaagaagaaaagt

SEQ ID NO: 4 - DNA, 62 bp, Artificial Sequence
  cT2
cccaaccctacccaccctcaagaaaaaaaagtgataattgttgtcgaagaagaaaaaaaatt

SEQ ID NO: 5 - RNA, 40 nt, Homo sapiens
ggguuggccaaaggagaaccucaagcuccuggccugaucc

SEQ ID NO: 6 - RNA, 39 nt, Homo sapiens
ggccuggaggaggucuuuggcagguccccucucgggaaa

SEQ ID NO: 7 - RNA, 1298 nt, Homo sapiens
agaauguucuuuuggccacugugaagccucaggaaggggcucggauugcucaaggacccaugggagagaggaggcuuugacugggcugccugccugugaggucucuggacuagagguccaacgcaguccagcugacaaggauggaauacgccaugaagucccuuagccuucucuaccccaagucccucuccaggcaugugucagugcguaccucuguggugacccagcagcugcugucggagcccagccccaaggcccccagggcccggcccugccgcguaagcacggcggaucgaagcgugaggaagggcaucauggcuuacagucuugaggaccuccuccucaagguccgggacacucugaugcuggcagacaagcccuucuuccuggugcuggaggaagauggcacaacuguagagacagaagaguacuuccaagcccuggcaggggauacaguguucaugguccuccagaaggggcagaaauggcagcccccaucagaacaggggacaaggcacccacugucccucucccauaagccugccaagaagauugauguggcccguguaacguuugaucuguacaagcugaacccacaggacuucauuggcugccugaacgugaaggcgacuuuuuaugauacauacucccuuuccuaugaucugcacugcuguggggccaagcgcaucaugaaggaagcuuuccgcugggcccucuucagcaugcaggccacaggccacguacugcuuggcaccuccuguuaccugcagcagcuccucgaugcuacggaggaagggcagccccccaagggcaaggccucaucccuuaucccgaccugucugaagauacugcagugaaagcccaaguccuuggaagcuuuccccagugaaggacugacugggggccucacgcuuaacugguagugcccacaagccuggcagcuguagagccgcgaaccuccccacaccucccucaccgcgcaggacccugagugaggaggaggagcuggaaaccugggguggguuggccaaaggagaaccucaagcuccuggccugauccagcuccuuccugcccaaggcagcuuagcccauccagacugguccugaagucugucccuccauuggcaugaagucugccccuuagcaaucuggccucgcaggcuguacuuucauggugcucucuaccuucuggcccccaucccggaacauuccugagugaauucgcaagcgcacuagcaugugauauuagggaguuugcaauaaauuauugaggcugauguaaaaaaaaaaaaaaaaaa

SEQ ID NO: 8 - RNA, 2642 nt, Homo sapiens
agcggagcgcggaggccgcugggacgcgguucagcucauucccugaggccggcccgcgucccgucaggcgccgcgcgggguuagcgcggggucagcggaggucagcgggggucagcagcagcggcuccgagggcgcggcggacgcaggauguacacgcugcugucgggcuuguacaaguacauguuucagaaggacgaguacugcauccugauccugggccuggacaaugcugggaagacgaccuuccuggagcagucgaaaacccgauuuaacaagaacuacaaggggaugagucuauccaaaaucaccaccaccgugggccuaaacaucggcacuguggaugugggaaaggcucggcucauguucugggacuuaggagggcaggaagagcugcagucuuugugggacaaguauuaugcggagugucacggcgucaucuacgucauugacuccaccgacgaggagaggcuggcugaguccaagcaggcguuugagaagguggugaccagcgaggcgcugugcgguguccccgucuuggugcuggccaacaagcaggauguggagacgugccucucaaucccugacaucaagacggccuucagcgacugcaccagcaagaucggcaggcgagauugccugacccaggccugcucggcccucacagggugagugggggcugcaccugcgggggcuuuggggaccgagaccccccgccucacacccgcugucuucacagcaaaggggugcgcgagggcaucgaguggauggugaagugugucgugcggaaugugcaccggccgccgcggcagagggacaucacguaggcgcagccgcgcugccgucgggacggcugguccccuggugcuggaggaguggccuccuguuggcucccaugcugcugaucugggggguggguuugcuuugcuuugggguucuucuauuuacuuuguuuucucgaagacaaacuuuccucuaugucuggaaaagcguaggcauccggaggcuuuggaggggagucuggcagcccggcuggcccaggcccugcagcggcagccuuuccacagggcgcagcggcggccuuucgaggcccuuucuggggggucugagggagaccugguugggaauuggggcuccagugcucaggcuggcuugggcugcaugaggacagcccugugggacccucgggagaccccguggcugucuccgccccaucgaggaggaggcccgucagccauggcugccaucuggcuucugcccugugaccccgugaccccgugaccccggaaguggucuggggcugaucuugccuugaggaagacccaggccauguucccaaaggccagcgggggcccuggauugugaugcagccucgggacagggcugaggccugcgggggaagaccuauaccccacgccugggccuggcuucaccucacccuaaucccccgggagggagcugacugaugcaaaaagcugagggggccugcugggaguggcuguuuuuaugccccagccccgcaaguuggggaguguuuguggggguccagagcccucccccagccaggagagaaccucccggagggguucucuguggggcccuguguccccugcucgggaguaaggcugguccugggguccucccugcacggaccccacugggccugccgagugcuguguucuuccucagucuggcugugggcaggagcggccugcccagugucacccagggugagugcaaaauaaagacggcgaguguggcucuguccaucccuucccuccuggaggguggaggcuccuggcuguuggacacggugaugguguuacugggcugcucaggggcuggugggcaggugaggggcuccccaggugggccuggagaguccaggcacucccuuccugcggaugugggaaggacaugggguccugggaggagcugcugggaaggggcaugagucaggguggggguggcgcagcagcugcggggcugugacucacaggagucgggcccuggaaguccccgcguccucuccaggggacccuguguguguucugcagguugguucccaggaccugggggggaccuccagccccgggaaccuggccgugcuggggaggcgaguggcuggugcagccccccgguugcucugggugcaucgggaggcuucagagccugccccagagagggagaagcuucacuucccggaaagcaugggaggccuggaggaggucuuuggcagguccccucucgggaaauccccugugaguugggagugggaggaauucauaagugggggguuagugugggccccggcgacuagggcuggccugagccccauccuguucuuccagcaaugauacccucccaggcccugacccucgcugagcuucaggggccccugccacgugccacagccacugggggcagagguggcacuccccacugauccucccagggagggucugucugagguaggggaagccccgggcagcaguucugauggcaggcagccugagggaucugggcacagcgggcggcucagguguccccggcugcccucccaguagcugugcaacuacaaccaguuuuaugaaaaagcuuuauaaaaauaagcuuuaagaaaccucaaaaaaaaaaaaaaaaa

SEQ ID NO: 9 - DNA, 40 bp, Homo sapiens
gggttggccaaaggagaacctcaagctcctggcctgatcc

SEQ ID NO: 10 - DNA, 1298 bp, Homo sapiens
agaatgttcttttggccactgtgaagcctcaggaaggggctcggattgctcaaggacccatgggagagaggaggctttgactgggctgcctgcctgtgaggtctctggactagaggtccaacgcagtccagctgacaaggatggaatacgccatgaagtcccttagccttctctaccccaagtccctctccaggcatgtgtcagtgcgtacctctgtggtgacccagcagctgctgtcggagcccagccccaaggcccccagggcccggccctgccgcgtaagcacggcggatcgaagcgtgaggaagggcatcatggcttacagtcttgaggacctcctcctcaaggtccgggacactctgatgctggcagacaagcccttcttcctggtgctggaggaagatggcacaactgtagagacagaagagtacttccaagccctggcaggggatacagtgttcatggtcctccagaaggggcagaaatggcagcccccatcagaacaggggacaaggcacccactgtccctctcccataagcctgccaagaagattgatgtggcccgtgtaacgtttgatctgtacaagctgaacccacaggacttcattggctgcctgaacgtgaaggcgactttttatgatacatactccctttcctatgatctgcactgctgtggggccaagcgcatcatgaaggaagctttccgctgggccctcttcagcatgcaggccacaggccacgtactgcttggcacctcctgttacctgcagcagctcctcgatgctacggaggaagggcagccccccaagggcaaggcctcatcccttatcccgacctgtctgaagatactgcagtgaaagcccaagtccttggaagctttccccagtgaaggactgactgggggcctcacgcttaactggtagtgcccacaagcctggcagctgtagagccgcgaacctccccacacctccctcaccgcgcaggaccctgagtgaggaggaggagctggaaacctggggtgggttggccaaaggagaacctcaagctcctggcctgatccagctccttcctgcccaaggcagcttagcccatccagactggtcctgaagtctgtccctccattggcatgaagtctgccccttagcaatctggcctcgcaggctgtactttcatggtgctctctaccttctggcccccatcccggaacattcctgagtgaattcgcaagcgcactagcatgtgatattagggagtttgcaataaattattgaggctgatgtaaaaaaaaaaaaaaaaaa

SEQ ID NO: 11 - DNA, 39 bp, Homo sapiens
ggcctggaggaggtctttggcaggtcccctctcgggaaa

SEQ ID NO: 12 - DNA, 2642 bp, Homo sapiens
agcggagcgcggaggccgctgggacgcggttcagctcattccctgaggccggcccgcgtcccgtcaggcgccgcgcggggttagcgcggggtcagcggaggtcagcgggggtcagcagcagcggctccgagggcgcggcggacgcaggatgtacacgctgctgtcgggcttgtacaagtacatgtttcagaaggacgagtactgcatcctgatcctgggcctggacaatgctgggaagacgaccttcctggagcagtcgaaaacccgatttaacaagaactacaaggggatgagtctatccaaaatcaccaccaccgtgggcctaaacatcggcactgtggatgtgggaaaggctcggctcatgttctgggacttaggagggcaggaagagctgcagtctttgtgggacaagtattatgcggagtgtcacggcgtcatctacgtcattgactccaccgacgaggagaggctggctgagtccaagcaggcgtttgagaaggtggtgaccagcgaggcgctgtgcggtgtccccgtcttggtgctggccaacaagcaggatgtggagacgtgcctctcaatccctgacatcaagacggccttcagcgactgcaccagcaagatcggcaggcgagattgcctgacccaggcctgctcggccctcacagggtgagtgggggctgcacctgcgggggctttggggaccgagaccccccgcctcacacccgctgtcttcacagcaaaggggtgcgcgagggcatcgagtggatggtgaagtgtgtcgtgcggaatgtgcaccggccgccgcggcagagggacatcacgtaggcgcagccgcgctgccgtcgggacggctggtcccctggtgctggaggagtggcctcctgttggctcccatgctgctgatctggggggtgggtttgctttgctttggggttcttctatttactttgttttctcgaagacaaactttcctctatgtctggaaaagcgtaggcatccggaggctttggaggggagtctggcagcccggctggcccaggccctgcagcggcagcctttccacagggcgcagcggcggcctttcgaggccctttctggggggtctgagggagacctggttgggaattggggctccagtgctcaggctggcttgggctgcatgaggacagccctgtgggaccctcgggagaccccgtggctgtctccgccccatcgaggaggaggcccgtcagccatggctgccatctggcttctgccctgtgaccccgtgaccccgtgaccccggaagtggtctggggctgatcttgccttgaggaagacccaggccatgttcccaaaggccagcgggggccctggattgtgatgcagcctcgggacagggctgaggcctgcgggggaagacctataccccacgcctgggcctggcttcacctcaccctaatcccccgggagggagctgactgatgcaaaaagctgagggggcctgctgggagtggctgtttttatgccccagccccgcaagttggggagtgtttgtgggggtccagagccctcccccagccaggagagaacctcccggaggggttctctgtggggccctgtgtcccctgctcgggagtaaggctggtcctggggtcctccctgcacggaccccactgggcctgccgagtgctgtgttcttcctcagtctggctgtgggcaggagcggcctgcccagtgtcacccagggtgagtgcaaaataaagacggcgagtgtggctctgtccatcccttccctcctggagggtggaggctcctggctgttggacacggtgatggtgttactgggctgctcaggggctggtgggcaggtgaggggctccccaggtgggcctggagagtccaggcactcccttcctgcggatgtgggaaggacatggggtcctgggaggagctgctgggaaggggcatgagtcagggtgggggtggcgcagcagctgcggggctgtgactcacaggagtcgggccctggaagtccccgcgtcctctccaggggaccctgtgtgtgttctgcaggttggttcccaggacctgggggggacctccagccccgggaacctggccgtgctggggaggcgagtggctggtgcagccccccggttgctctgggtgcatcgggaggcttcagagcctgccccagagagggagaagcttcacttcccggaaagcatgggaggcctggaggaggtctttggcaggtcccctctcgggaaatcccctgtgagttgggagtgggaggaattcataagtggggggttagtgtgggccccggcgactagggctggcctgagccccatcctgttcttccagcaatgataccctcccaggccctgaccctcgctgagcttcaggggcccctgccacgtgccacagccactgggggcagaggtggcactccccactgatcctcccagggagggtctgtctgaggtaggggaagccccgggcagcagttctgatggcaggcagcctgagggatctgggcacagcgggcggctcaggtgtccccggctgccctcccagtagctgtgcaactacaaccagttttatgaaaaagctttataaaaataagctttaagaaacctcaaaaaaaaaaaaaaaaa

SEQ ID NO: 13 - DNA, 74 bp, Artificial Sequence
  cT1-9bp
ccccaaaaaggagcttgaggttctcctttaaaggagagaaagaagctgttgtattgttgtcgaagaagaaaagt

SEQ ID NO: 14 - DNA, 34 bp, Artificial Sequence
  CS-mir-21ca
aaaggagaacctcaagctcctcagtctgataagc

SEQ ID NO: 15 - RNA, 24 nt, Homo sapiens
uagcuuaucagacugauguugaca

SEQ ID NO: 16 - RNA, 22 nt, Homo sapiens
uagcuuaucagacugauguuga

SEQ ID NO: 17 - RNA, 23 nt, Homo sapiens
agcuacauugucugcuggguuuc

SEQ ID NO: 18 - DNA, 67 bp, Artificial Sequence
  cT1-mir-21ca
ctgtcaacaggagcttgaggttctcctttaaaaagaagctgttgtattgttgtcgaagaagaaaagt

SEQ ID NO: 19 - DNA, 17 bp, Artificial Sequence
  P1-thr
tggttggaaattttttg

SEQ ID NO: 20 - DNA, 35 bp, Artificial Sequence
  CS-mir-13b
aaaggagaacctcaagctccaaaatggctgtgata

SEQ ID NO: 21 - RNA, 22 nt, Homo sapiens
uaucacagccauuuugaugagu

SEQ ID NO: 22 - RNA, 22 nt, Homo sapiens
uaucacagccauuuugacgagu

SEQ ID NO: 23 - DNA, 66 bp, Artificial Sequence
  cT1-mir-13b
cactcatcggagcttgaggttctcctttaaaaagaagctgttgtattgttgtcgaagaagaaaagt

SEQ ID NO: 24 - DNA, 31 bp, Artificial Sequence
  CS-thr
aaaggagaacctcaagctcctttggttggtg

SEQ ID NO: 25 - DNA, 67 bp, Artificial Sequence
  cT1-thr
cccaaaaaaggagcttgaggttctcctttaaaaagaagctgttgtattgttgtcgaagaagaaaagt

SEQ ID NO: 26 - DNA, 37 bp, Artificial Sequence
  CS-str
aaaggagaacctcaagctccggcaccacggucggauc

SEQ ID NO: 27 - DNA, 28 bp, Artificial Sequence
  P1-str
gaucgcauuuggacuucugccttttttg